European Patent Specification EP 3 490 585 B1, published May 17, 2023. Title: IMMUNOMODULATORY POLYPEPTIDES AND RELATED COMPOSITIONS AND METHODS. Applicant: Juno Therapeutics, Inc. Hauskins, Collin Ebens, Allen. Application Not Yet Assigned. The sequence listing filed with the application follows.

SEQUENCE LISTING (118 sequences)

SEQ ID NO: 1 - protein, 518 aa, Artificial Sequence
  Sc IL-12 G4S(3)
IWELKKDVYVVELDWYPDAPGEMVVLTCDTPEEDGITWTLDQSSEVLGSGKTLTIQVKEFGDAGQYTCHKGGEVLSHSLLLLHKKEDGIWSTDILKDQKEPKNKTFLRCEAKNYSGRFTCWWLTTISTDLTFSVKSSRGSSDPQGVTCGAATLSAERVRGDNKEYEYSVECQEDSACPAAEESLPIEVMVDAVHKLKYENYTSSFFIRDIIKPDPPKNLQLKPLKNSRQVEVSWEYPDTWSTPHSYFSLTFCVQVQGKSKREKKDRVFTDKTSATVICRKNASISVRAQDRYYSSSWSEWASVPCSGGGGSGGGGSGGGGSRNLPVATPDPGMFPCLHHSQNLLRAVSNMLQKARQTLEFYPCTSEEIDHEDITKDKTSTVEACLPLELTKNESCLNSRETSFITNGSCLASRKTSFMMALCLSSIYEDLKMYQVEFKTMNAKLLMDPKRQIFLDQNMLAVIDELMQALNFNSETVPQKSSLEEPDFYKTKIKLCILLHAFRIRAVTIDRVMSYLNAS

SEQ ID NO: 2 - protein, 523 aa, Artificial Sequence
  Sc IL-12 HBP BMP4
IWELKKDVYVVELDWYPDAPGEMVVLTCDTPEEDGITWTLDQSSEVLGSGKTLTIQVKEFGDAGQYTCHKGGEVLSHSLLLLHKKEDGIWSTDILKDQKEPKNKTFLRCEAKNYSGRFTCWWLTTISTDLTFSVKSSRGSSDPQGVTCGAATLSAERVRGDNKEYEYSVECQEDSACPAAEESLPIEVMVDAVHKLKYENYTSSFFIRDIIKPDPPKNLQLKPLKNSRQVEVSWEYPDTWSTPHSYFSLTFCVQVQGKSKREKKDRVFTDKTSATVICRKNASISVRAQDRYYSSSWSEWASVPCSGGGGSRKKNPNCRRHGGGGSRNLPVATPDPGMFPCLHHSQNLLRAVSNMLQKARQTLEFYPCTSEEIDHEDITKDKTSTVEACLPLELTKNESCLNSRETSFITNGSCLASRKTSFMMALCLSSIYEDLKMYQVEFKTMNAKLLMDPKRQIFLDQNMLAVIDELMQALNFNSETVPQKSSLEEPDFYKTKIKLCILLHAFRIRAVTIDRVMSYLNAS

SEQ ID NO: 3 - protein, 528 aa, Artificial Sequence
  Sc IL-12 HBP FBN
IWELKKDVYVVELDWYPDAPGEMVVLTCDTPEEDGITWTLDQSSEVLGSGKTLTIQVKEFGDAGQYTCHKGGEVLSHSLLLLHKKEDGIWSTDILKDQKEPKNKTFLRCEAKNYSGRFTCWWLTTISTDLTFSVKSSRGSSDPQGVTCGAATLSAERVRGDNKEYEYSVECQEDSACPAAEESLPIEVMVDAVHKLKYENYTSSFFIRDIIKPDPPKNLQLKPLKNSRQVEVSWEYPDTWSTPHSYFSLTFCVQVQGKSKREKKDRVFTDKTSATVICRKNASISVRAQDRYYSSSWSEWASVPCSGGGGSKNNQKSEPLIGRKKTGGGGSRNLPVATPDPGMFPCLHHSQNLLRAVSNMLQKARQTLEFYPCTSEEIDHEDITKDKTSTVEACLPLELTKNESCLNSRETSFITNGSCLASRKTSFMMALCLSSIYEDLKMYQVEFKTMNAKLLMDPKRQIFLDQNMLAVIDELMQALNFNSETVPQKSSLEEPDFYKTKIKLCILLHAFRIRAVTIDRVMSYLNAS

SEQ ID NO: 4 - protein, 529 aa, Artificial Sequence
  Sc IL-12 HGFBP
IWELKKDVYVVELDWYPDAPGEMVVLTCDTPEEDGITWTLDQSSEVLGSGKTLTIQVKEFGDAGQYTCHKGGEVLSHSLLLLHKKEDGIWSTDILKDQKEPKNKTFLRCEAKNYSGRFTCWWLTTISTDLTFSVKSSRGSSDPQGVTCGAATLSAERVRGDNKEYEYSVECQEDSACPAAEESLPIEVMVDAVHKLKYENYTSSFFIRDIIKPDPPKNLQLKPLKNSRQVEVSWEYPDTWSTPHSYFSLTFCVQVQGKSKREKKDRVFTDKTSATVICRKNASISVRAQDRYYSSSWSEWASVPCSGGGGSVWNWVCFRDVGCDWVLGGGGSRNLPVATPDPGMFPCLHHSQNLLRAVSNMLQKARQTLEFYPCTSEEIDHEDITKDKTSTVEACLPLELTKNESCLNSRETSFITNGSCLASRKTSFMMALCLSSIYEDLKMYQVEFKTMNAKLLMDPKRQIFLDQNMLAVIDELMQALNFNSETVPQKSSLEEPDFYKTKIKLCILLHAFRIRAVTIDRVMSYLNAS

SEQ ID NO: 5 - protein, 521 aa, Artificial Sequence
  Sc IL-12 EGFRBP
IWELKKDVYVVELDWYPDAPGEMVVLTCDTPEEDGITWTLDQSSEVLGSGKTLTIQVKEFGDAGQYTCHKGGEVLSHSLLLLHKKEDGIWSTDILKDQKEPKNKTFLRCEAKNYSGRFTCWWLTTISTDLTFSVKSSRGSSDPQGVTCGAATLSAERVRGDNKEYEYSVECQEDSACPAAEESLPIEVMVDAVHKLKYENYTSSFFIRDIIKPDPPKNLQLKPLKNSRQVEVSWEYPDTWSTPHSYFSLTFCVQVQGKSKREKKDRVFTDKTSATVICRKNASISVRAQDRYYSSSWSEWASVPCSGGGGSSVDNPHVCGGGGSRNLPVATPDPGMFPCLHHSQNLLRAVSNMLQKARQTLEFYPCTSEEIDHEDITKDKTSTVEACLPLELTKNESCLNSRETSFITNGSCLASRKTSFMMALCLSSIYEDLKMYQVEFKTMNAKLLMDPKRQIFLDQNMLAVIDELMQALNFNSETVPQKSSLEEPDFYKTKIKLCILLHAFRIRAVTIDRVMSYLNAS

SEQ ID NO: 6 - protein, 760 aa, Artificial Sequence
  Sc IL-12 Anti EPCAM
IWELKKDVYVVELDWYPDAPGEMVVLTCDTPEEDGITWTLDQSSEVLGSGKTLTIQVKEFGDAGQYTCHKGGEVLSHSLLLLHKKEDGIWSTDILKDQKEPKNKTFLRCEAKNYSGRFTCWWLTTISTDLTFSVKSSRGSSDPQGVTCGAATLSAERVRGDNKEYEYSVECQEDSACPAAEESLPIEVMVDAVHKLKYENYTSSFFIRDIIKPDPPKNLQLKPLKNSRQVEVSWEYPDTWSTPHSYFSLTFCVQVQGKSKREKKDRVFTDKTSATVICRKNASISVRAQDRYYSSSWSEWASVPCSGGGGSQVQLVQSGAEVKKPGSSVKVSCKASGGTFSSYAISVVVRQAPGQGLEWMGGIIPIFGTANYAQKFQGRVTITADESTSTAYMELSSLRSEDTAVYYCARGLLWNYWGQGTLVTVSSKLSGSASAPKLEEGEFSEARVETTLTQSPATLSVSPGERATLSCRASQSVSSNLAVVYQQKPGQAPRLLIYGASTRATGIPARFSGSGSGTEFTLTISSLQSEDFAVYYCQQYNNWPPGFTFGPGTKVDIKGGGGSRNLPVATPDPGMFPCLHHSQNLLRAVSNMLQKARQTLEFYPCTSEEIDHEDITKDKTSTVEACLPLELTKNESCLNSRETSFITNGSCLASRKTSFMMALCLSSIYEDLKMYQVEFKTMNAKLLMDPKRQIFLDQNMLAVIDELMQALNFNSETVPQKSSLEEPDFYKTKIKLCILLHAFRIRAVTIDRVMSYLNAS

SEQ ID NO: 7 - protein, 5 aa, Artificial Sequence
  G4S linker
GGGGS

SEQ ID NO: 8 - protein, 10 aa, Artificial Sequence
  G4S(2) linker
GGGGSGGGGS

SEQ ID NO: 9 - protein, 15 aa, Artificial Sequence
  G4S(3) linker
GGGGSGGGGSGGGGS

SEQ ID NO: 10 - protein, 197 aa, Artificial Sequence
  IL-12 p35
RNLPVATPDPGMFPCLHHSQNLLRAVSNMLQKARQTLEFYPCTSEEIDHEDITKDKTSTVEACLPLELTKNESCLNSRETSFITNGSCLASRKTSFMMALCLSSIYEDLKMYQVEFKTMNAKLLMDPKRQIFLDQNMLAVIDELMQALNFNSETVPQKSSLEEPDFYKTKIKLCILLHAFRIRAVTIDRVMSYLNAS

SEQ ID NO: 11 - protein, 306 aa, Artificial Sequence
  IL-12 p40
IWELKKDVYVVELDWYPDAPGEMVVLTCDTPEEDGITWTLDQSSEVLGSGKTLTIQVKEFGDAGQYTCHKGGEVLSHSLLLLHKKEDGIWSTDILKDQKEPKNKTFLRCEAKNYSGRFTCWWLTTISTDLTFSVKSSRGSSDPQGVTCGAATLSAERVRGDNKEYEYSVECQEDSACPAAEESLPIEVMVDAVHKLKYENYTSSFFIRDIIKPDPPKNLQLKPLKNSRQVEVSWEYPDTWSTPHSYFSLTFCVQVQGKSKREKKDRVFTDKTSATVICRKNASISVRAQDRYYSSSWSEWASVPCS

SEQ ID NO: 12 - protein, 22 aa, Artificial Sequence
  IL-12p40 signal sequence
MCHQQLVISWFSLVFLASPLVA

SEQ ID NO: 13 - protein, 10 aa, Artificial Sequence
  Heparin binding peptide, BMP4
RKKNPNCRRH

SEQ ID NO: 14 - protein, 15 aa, Artificial Sequence
  Heparin binding peptide, fibronectin
KNNQKSEPLIGRKKT

SEQ ID NO: 15 - protein, 16 aa, Artificial Sequence
  HGF binding peptide
VWNWVCFRDVGCDWVL

SEQ ID NO: 16 - protein, 8 aa, Artificial Sequence
  EGFRBP
SVDNPHVC

SEQ ID NO: 17 - protein, 247 aa, Artificial Sequence
  Anti-EPCAM scFv
QVQLVQSGAEVKKPGSSVKVSCKASGGTFSSYAISVVVRQAPGQGLEWMGGIIPIFGTANYAQKFQGRVTITADESTSTAYMELSSLRSEDTAVYYCARGLLWNYWGQGTLVTVSSKLSGSASAPKLEEGEFSEARVETTLTQSPATLSVSPGERATLSCRASQSVSSNLAVVYQQKPGQAPRLLIYGASTRATGIPARFSGSGSGTEFTLTISSLQSEDFAVYYCQQYNNWPPGFTFGPGTKVDIK

SEQ ID NO: 18 - protein, 17 aa, Artificial Sequence
  CD33 signal sequence
MPLLLLLPLLWAGALAM

SEQ ID NO: 19 - protein, 22 aa, Artificial Sequence
  IL-12 p35 signal sequence
MCPARSLLLVATLVLLDHLSLA

SEQ ID NO: 20 - protein, 6 aa, Artificial Sequence
  6x His-tag
HHHHHH

SEQ ID NO: 21 - protein, 8 aa, Artificial Sequence
  Strep-tag(r) II
WSHPQFEK

SEQ ID NO: 22 - protein, 21 aa, Artificial Sequence
  linker
KLSGSASAPKLEEGEFSEARV

SEQ ID NO: 23 - protein, 18 aa, Artificial Sequence
  linker
GSTSGSGKPGSGEGSTKG

SEQ ID NO: 24 - protein, 116 aa, Artificial Sequence
  Anti-EPCAM
QVQLVQSGAEVKKPGSSVKVSCKASGGTFSSYAISVVVRQAPGQGLEWMGGIIPIFGTANYAQKFQGRVTITADESTSTAYMELSSLRSEDTAVYYCARGLLWNYWGQGTLVTVSS

SEQ ID NO: 25 - protein, 110 aa, Artificial Sequence
  Anti-EPCAM variable heavy (VH)
ETTLTQSPATLSVSPGERATLSCRASQSVSSNLAVVYQQKPGQAPRLLIYGASTRATGIPARFSGSGSGTEFTLTISSLQSEDFAVYYCQQYNNWPPGFTFGPGTKVDIK

SEQ ID NO: 26 - protein, 7 aa, Artificial Sequence
  VEGF binding peptide
ATWLPPR

SEQ ID NO: 27 - protein, 23 aa, Artificial Sequence
  VEGFR binding peptide
ITMQCGIHQGQHPKIRMICEMSF

SEQ ID NO: 28 - protein, 8 aa, Artificial Sequence
  bovine origin heparin binding peptide
WQPPRARI

SEQ ID NO: 29 - protein, 25 aa, Artificial Sequence
  Linker (GGGGS)n; n is 1 to 5
  VARIANT (6)..(10): (Xaa Xaa Xaa Xaa Xaa) = (Gly Gly Gly Gly Ser) or null
  VARIANT (11)..(15): (Xaa Xaa Xaa Xaa Xaa) = (Gly Gly Gly Gly Ser) or null
  VARIANT (16)..(20): (Xaa Xaa Xaa Xaa Xaa) = (Gly Gly Gly Gly Ser) or null
  VARIANT (21)..(25): (Xaa Xaa Xaa Xaa Xaa) = (Gly Gly Gly Gly Ser) or null
GGGGSXXXXXXXXXXXXXXXXXXXX

SEQ ID NO: 30 - protein, 133 aa, Homo sapiens
  misc_feature: IL-15
GIHVFILGCFSAGLPKTEANWVNVISDLKKIEDLIQSMHIDATLYTESDVHPSCKVTAMKCFLLELQVISLESGDASIHDTVENLIILANNSLSSNGNVTESGCKECEELEEKNIKEFLQSFVHIVQMFINTS

SEQ ID NO: 31 - protein, 133 aa, Homo sapiens [sequence omitted]

SEQ ID NO: 32 - protein, 193 aa, Homo sapiens
  misc_feature: IL-19
MAAEPVEDNCINFVAMKFIDNTLYFIAEDDENLESDYFGKLESKLSVIRNLNDQVLFIDQGNRPLFEDMTDSDCRDNAPRTIFIISMYKDSQPRGMAVTISVKCEKISTLSCENKIISFKEMNPPDNIKDTKSDIIFFQRSVPGHDNKMQFESSSYEGYFLACEKERDLFKLILKKEDELGDRSIMFTVQNED

SEQ ID NO: 33 - protein, 127 aa, Homo sapiens [sequence omitted]

SEQ ID NO: 34 - protein, 152 aa, Homo sapiens
  misc_feature: IL-7
DCDIEGKDGKQYESVLMVSIDQLLDSMKEIGSNCLNNEFNFFKRHICDANKEGMFLFRAARKLRQFLKMNSTGDFDLHLLKVSEGTTILLNCTGQVKGRKPAALGEAQPTKSLEENKSLKEQKKLNDLCFLKRLLQEIKTCWNKILMGTKEH

SEQ ID NO: 35 - protein, 133 aa, Homo sapiens [sequence omitted]

SEQ ID NO: 36 - protein, 166 aa, Homo sapiens
  misc_feature: IFN alpha-1/13
CDLPETHSLDNRRTLMLLAQMSRISPSSCLMDRHDFGFPQEEFDGNQFQKAPAISVLHELIQQIFNLFTTKDSSAAWDEDLLDKFCTELYQQLNDLEACVMQEERVGETPLMNADSILAVKKYFRRITLYLTEKKYSPCAWEVVRAEIMRSLSLSTNLQERLRRKE

SEQ ID NO: 37 - protein, 165 aa, Homo sapiens
  misc_feature: IFN alpha-2
CDLPQTHSLGSRRTLMLLAQMRKISLFSCLKDRHDFGFPQEEFGNQFQKAETIPVLHEMIQQIFNLFSTKDSSAAWDETLLDKFYTELYQQLNDLEACVIQGVGVTETPLMKEDSILAVRKYFQRITLYLKEKKYSPCAWEVVRAEIMRSFSLSTNLQESLRSKE

SEQ ID NO: 38 - protein, 166 aa, Homo sapiens
  misc_feature: IFN alpha-4
CDLPQTHSLGNRRALILLAQMGRISHFSCLKDRHDFGFPEEEFDGHQFQKAQAISVLHEMIQQTFNLFSTEDSSAAWEQSLLEKFSTELYQQLNDLEACVIQEVGVEETPLMNEDSILAVRKYFQRITLYLTEKKYSPCAWEVVRAEIMRSLSFSTNLQKRLRRKD

SEQ ID NO: 39 - protein, 168 aa, Homo sapiens
  misc_feature: IFN alpha-5
LGCDLPQTHSLSNRRTLMIMAQMGRISPFSCLKDRHDFGFPQEEFDGNQFQKAQAISVLHEMIQQTFNLFSTKDSSATWDETLLDKFYTELYQQLNDLEACMMQEVGVEDTPLMNVDSILTVRKYFQRITLYLTEKKYSPCAWEVVRAEIMRSFSLSANLQERLRRKE

SEQ ID NO: 40 - protein, 169 aa, Homo sapiens
  misc_feature: IFN alpha-6
SLDCDLPQTHSLGHRRTMMLLAQMRRISLFSCLKDRHDFRFPQEEFDGNQFQKAEAISVLHEVIQQTFNLFSTKDSSVAWDERLLDKLYTELYQQLNDLEACVMQEVWVGGTPLMNEDSILAVRKYFQRITLYLTEKKYSPCAWEVVRAEIMRSFSSSRNLQERLRRKE

SEQ ID NO: 41 - protein, 166 aa, Homo sapiens
  misc_feature: IFN alpha-7
CDLPQTHSLRNRRALILLAQMGRISPFSCLKDRHEFRFPEEEFDGHQFQKTQAISVLHEMIQQTFNLFSTEDSSAAWEQSLLEKFSTELYQQLNDLEACVIQEVGVEETPLMNEDFILAVRKYFQRITLYLMEKKYSPCAWEVVRAEIMRSFSFSTNLKKGLRRKD

SEQ ID NO: 42 - protein, 166 aa, Homo sapiens
  misc_feature: IFN alpha-8
CDLPQTHSLGNRRALILLAQMRRISPFSCLKDRHDFEFPQEEFDDKQFQKAQAISVLHEMIQQTFNLFSTKDSSAALDETLLDEFYIELDQQLNDLESCVMQEVGVIESPLMYEDSILAVRKYFQRITLYLTEKKYSSCAWEVVRAEIMRSFSLSINLQKRLKSKE

SEQ ID NO: 43 - protein, 166 aa, Homo sapiens
  misc_feature: IFN alpha-10
CDLPQTHSLGNRRALILLGQMGRISPFSCLKDRHDFRIPQEEFDGNQFQKAQAISVLHEMIQQTFNLFSTEDSSAAWEQSLLEKFSTELYQQLNDLEACVIQEVGVEETPLMNEDSILAVRKYFQRITLYLIERKYSPCAWEVVRAEIMRSLSFSTNLQKRLRRKD

SEQ ID NO: 44 - protein, 166 aa, Homo sapiens
  misc_feature: IFN alpha-14
CNLSQTHSLNNRRTLMLMAQMRRISPFSCLKDRHDFEFPQEEFDGNQFQKAQAISVLHEMMQQTFNLFSTKNSSAAWDETLLEKFYIELFQQMNDLEACVIQEVGVEETPLMNEDSILAVKKYFQRITLYLMEKKYSPCAWEVVRAEIMRSLSFSTNLQKRLRRKD

SEQ ID NO: 45 - protein, 166 aa, Homo sapiens
  misc_feature: IFN alpha-16
CDLPQTHSLGNRRALILLAQMGRISHFSCLKDRYDFGFPQEVFDGNQFQKAQAISAFHEMIQQTFNLFSTKDSSAAWDETLLDKFYIELFQQLNDLEACVTQEVGVEEIALMNEDSILAVRKYFQRITLYLMGKKYSPCAWEVVRAEIMRSFSFSTNLQKGLRRKD

SEQ ID NO: 46 - protein, 166 aa, Homo sapiens
  misc_feature: IFN alpha-17
CDLPQTHSLGNRRALILLAQMGRISPFSCLKDRHDFGLPQEEFDGNQFQKTQAISVLHEMIQQTFNLFSTEDSSAAWEQSLLEKFSTELYQQLNNLEACVIQEVGMEETPLMNEDSILAVRKYFQRITLYLTEKKYSPCAWEVVRAEIMRSLSFSTNLQKILRRKD

SEQ ID NO: 47 - protein, 166 aa, Homo sapiens
  misc_feature: IFN alpha-21
CDLPQTHSLGNRRALILLAQMGRISPFSCLKDRHDFGFPQEEFDGNQFQKAQAISVLHEMIQQTFNLFSTKDSSATWEQSLLEKFSTELNQQLNDLEACVIQEVGVEETPLMNVDSILAVKKYFQRITLYLTEKKYSPCAWEVVRAEIMRSFSLSKIFQERLRRKE

SEQ ID NO: 48 - protein, 166 aa, Homo sapiens
  misc_feature: IFN beta-1
MSYNLLGFLQRSSNFQCQKLLWQLNGRLEYCLKDRMNFDIPEEIKQLQQFQKEDAALTIYEMLQNIFAIFRQDSSSTGWNETIVENLLANVYHQINHLKTVLEEKLEKEDFTRGKLMSSLHLKRYYGRILHYLKAKEYSHCAWTIVRVEILRNFYFINRLTGYLRN

SEQ ID NO: 49 - protein, 143 aa, Homo sapiens
  misc_feature: IFN gamma
QDPYVKEAENLKKYFNAGHSDVADNGTLFLGILKNWKEESDRKIMQSQIVSFYFKLFKNFKDDQSIQKSVETIKEDMNVKFFNSNKKKRDDFEKLTNYSVTDLNVQRKAIHELIQVMAELSPAAKTGKRKRSQMLFRGRRASQ

SEQ ID NO: 50 - protein, 132 aa, Homo sapiens
  misc_feature: IL-17A
GITIPRNPGCPNSEDKNFPRTVMVNLNIHNRNTNTNPKRSSDYYNRSTSPWNLHRNEDPERYPSVIWEAKCRHLGCINADGNVDYHMNSVPIQQEILVLRREPPHCPNSFRLEKILVSVGCTCVTPIVHHVA

SEQ ID NO: 51 - protein, 133 aa, Homo sapiens [sequence omitted]

SEQ ID NO: 52 - protein, 170 aa, Homo sapiens
  misc_feature: IL-23 alpha (p19)
RAVPGGSSPAWTQCQQLSQKLCTLAWSAHPLVGHMDLREEGDEETTNDVPHIQCGDGCDPQGLRDNSQFCLQRIHQGLIFYEKLLGSDIFTGEPSLLPDSPVGQLHASLLGLSQLLQPEGHHWETQQIPSLSPSQPWQRLLLRFKILRSLQAFVAVAARVFAHGAATLSP

SEQ ID NO: 53 - protein, 133 aa, Homo sapiens
  misc_feature: IL-3
APMTQTTPLKTSWVNCSNMIDEIITHLKQPPLPLLDFNNLNGEDQDILMENNLRRPNLEAFNRAVKSLQNASAIESILKNLLPCLPLATAAPTRHPIHIKDGDWNEFRRKLTFYLKTLENAQAQQTTLSLAIF

SEQ ID NO: 54 - protein, 129 aa, Homo sapiens [sequence omitted]

SEQ ID NO: 55 - protein, 115 aa, Homo sapiens
IPTEIPTSALVKETLALLSTHRTLLIANETLRIPVPVHKNHQLCTEEIFQGIGTLESQTVQGGTVERLFKNLSLIKKYIDGQKKKCGEERRRVNQFLDYLQEFLGVMNTEWIIES

SEQ ID NO: 56 - protein, 183 aa, Homo sapiens
  misc_feature: IL-6
VPPGEDSKDVAAPHRQPLTSSERIDKQIRYILDGISALRKETCNKSNMCESSKEALAENNLNLPKMAEKDGCFQSGFNEETCLVKIITGLLEFEVYLEYLQNRFESSEEQARAVQMSTKVLIQFLQKKAKNLDAITTPDPTTNASLLTKLQAQNQWLQDMTTHLILRSFKEFLQSSLRALRQM

SEQ ID NO: 57 - protein, 126 aa, Homo sapiens
  misc_feature: IL-9
QGCPTLAGILDINFLINKMQEDPASKCHCSANVTSCLCLGIPSDNCTRPCFSERLSQMTNTTMQTRYPLIFSRVKKSVEVLKNNKCPYFSCEQPCNQTTAGNALTFLKSLLEIFQKEKMRGMRGKI

SEQ ID NO: 58 - protein, 178 aa, Homo sapiens
  misc_feature: IL-11
PGPPPGPPRVSPDPRAELDSTVLLTRSLLADTRQLAAQLRDKFPADGDHNLDSLPTLAMSAGALGALQLPGVLTRLRADLLSYLRHVQWLRRAGGSSLKTLEPELGTLQARLDRLLRRLQLLMSRLALPQPPPDPPAPPLAPPSSAWGGIRAAHAILGGLHLTLDWAVRGLLLLKTRL

SEQ ID NO: 59 - protein, 122 aa, Homo sapiens
  misc_feature: IL-13
LTCLGGFASPGPVPPSTALRELIEELVNITQNQKAPLCNGSMVWSINLTAGMYCAALESLINVSGCSAIEKTQRMLSGFCPHKVSAGQFSSLHVRDTKIEVAQFVKDLLLHLKKLFREGRFN

SEQ ID NO: 60 - protein, 215 aa, Homo sapiens
  misc_feature: IL-27 alpha (p28)
FPRPPGRPQLSLQELRREFTVSLHLARKLLSEVRGQAHRFAESHLPGVNLYLLPLGEQLPDVSLTFQAWRRLSDPERLCFISTTLQPFHALLGGLGTQGRWTNMERMQLWAMRLDLRDLQRHLRFQVLAAGFNLPEEEEEEEEEEEEERKGLLPGALGSALQGPAQVSWPQLLSTYRLLHSLELVLSRAVRELLLLSKAGHSVWPLGFPTLSPQP

SEQ ID NO: 61 - protein, 209 aa, Homo sapiens
  misc_feature: IL-27 beta (EBI3), IL-35 beta
RKGPPAALTLPRVQCRASRYPIAVDCSWTLPPAPNSTSPVSFIATYRLGMAARGHSWPCLQQTPTSTSCTITDVQLFSMAPYVLNVTAVHPWGSSSSFVPFITEHIIKPDPPEGVRLSPLAERQLQVQWEPPGSWPFPEIFSLKYWIRYKRQGAARFHRVGPIEATSFILRAVRPRARYYVQVAAQDLTDYGELSDWSLPATATMSLGK

SEQ ID NO: 62 - protein, 166 aa, Homo sapiens
  misc_feature: Erythropoietin
APPRLICDSRVLERYLLEAKEAENITTGCAEHCSLNENITVPDTKVNFYAWKRMEVGQQAVEVWQGLALLSEAVLRGQALLVNSSQPWEPLQLHVDKAVSGLRSLTTLLRALGAQKEAISPPDAASAAPLRTITADTFRKLFRVYSNFLRGKLKLYTGEACRTGDR

SEQ ID NO: 63 - protein, 178 aa, Homo sapiens
  misc_feature: G-CSF
ATPLGPASSLPQSFLLKCLEQVRKIQGDGAALQEKLVSECATYKLCHPEELVLLGHSLGIPWAPLSSCPSQALQLAGCLSQLHSGLFLYQGLLQALEGISPELGPTLDTLQLDVADFATTIWQQMEELGMAPALQPTQGAMPAFASAFQRRAGGVLVASHLQSFLEVSYRVLRHLAQP

SEQ ID NO: 64 - protein, 191 aa, Homo sapiens [sequence omitted]

SEQ ID NO: 65 - protein, 199 aa, Homo sapiens
  misc_feature: Prolactin
LPICPGGAARCQVTLRDLFDRAVVLSHYIHNLSSEMFSEFDKRYTHGRGFITKAINSCHTSSLATPEDKEQAQQMNQKDFLSLIVSILRSWNEPLYHLVTEVRGMQEAPEAILSKAVEIEEQTKRLLEGMELIVSQVHPETKENEIYPVWSGLPSLQMADEESRLSAYYNLLHCLRRDSHKIDNYLKLLKCRIIHNNNC

SEQ ID NO: 66 - protein, 227 aa, Homo sapiens
  misc_feature: Oncostatin M
AAIGSCSKEYRVLLGQLQKQTDLMQDTSRLLDPYIRIQGLDVPKLREHCRERPGAFPSEETLRGLGRRGFLQTLNATLGCVLHRLADLEQRLPKAQDLERSGLNIEDLEKLQMARPNILGLRNNIYCMAQLLDNSDTAEPTKAGRGASQPPTPTPASDAFQRKLEGCRFLHGYHRFMHSVGRVFSKWGESPNRSRRHSPHQALRKGVRRTRPSRKGKRLMTRGQLPR

SEQ ID NO: 67 - protein, 180 aa, Homo sapiens
  misc_feature: Leukemia inhibitory factor
SPLPITPVNATCAIRHPCHNNLMNQIRSQLAQLNGSANALFILYYTAQGEPFPNNLDKLCGPNVTDFPPFHANGTEKAKLVELYRIVVYLGTSLGNITRDQKILNPSALSLHSKLNATADILRGLLSNVLCRLCSKYHVGHVDVTYGPDTSGKDVFQKKKLGCQLLGKYKQIIAVLAQAF

SEQ ID NO: 68 - protein, 146 aa, Homo sapiens
  misc_feature: IL-22
APISSHCRLDKSNFQQPYITNRTFMLAKEASLADNNTDVRLIGEKLFHGVSMSERCYLMKQVLNFTLEEVLFPQSDRFQPYMQEVVPFLARLSNRLSTCHIEGDDLHIQRNVQKLKDTVKKLGESGEIKAIGELDLLFMSLRNACI

SEQ ID NO: 69 - protein, 160 aa, Homo sapiens
  misc_feature: IL-10
SPGQGTQSENSCTHFPGNLPNMLRDLRDAFSRVKTFFQMKDQLDNLLLKESLLEDFKGYLGCQALSEMIQFYLEEVMPQAENQDPDIKAHVNSLGENLKTLRLRLRRCHRFLPCENKSKAVEQVKNAFNKLQEKGIYKAMSEFDIFINYIEAYMTMKIRN

SEQ ID NO: 70 - protein, 12 aa, Artificial Sequence
  spacer (IgG4hinge)
ESKYGPPCPPCP

SEQ ID NO: 71 - protein, 36 aa, Artificial Sequence
  spacer (IgG4hinge)
GAATCTAAGTACGGACCGCCCTGCCCCCCTTGCCCT

SEQ ID NO: 72 - protein, 119 aa, Artificial Sequence
  Hinge-CH3 spacer
ESKYGPPCPPCPGQPREPQVYTLPPSQEEMTKNQVSLTCLVKGFYPSDIAVEWESNGQPENNYKTTPPVLDSDGSFFLYSRLTVDKSRWQEGNVFSCSVMHEALHNHYTQKSLSLSLGK

SEQ ID NO: 73 - protein, 229 aa, Artificial Sequence
  Hinge-CH2-CH3 spacer
ESKYGPPCPPCPAPEFLGGPSVFLFPPKPKDTLMISRTPEVTCVVVDVSQEDPEVQFNWYVDGVEVHNAKTKPREEQFNSTYRVVSVLTVLHQDWLNGKEYKCKVSNKGLPSSIEKTISKAKGQPREPQVYTLPPSQEEMTKNQVSLTCLVKGFYPSDIAVEWESNGQPENNYKTTPPVLDSDGSFFLYSRLTVDKSRWQEGNVFSCSVMHEALHNHYTQKSLSLSLGK

SEQ ID NO: 74 - protein, 282 aa, Artificial Sequence
  IgD-hinge-Fc
RWPESPKAQASSVPTAQPQAEGSLAKATTAPATTRNTGRGGEEKKKEKEKEEQEERETKTPECPSHTQPLGVYLLTPAVQDLWLRDKATFTCFVVGSDLKDAHLTWEVAGKVPTGGVEEGLLERHSNGSQSQHSRLTLPRSLWNAGTSVTCTLNHPSLPPQRLMALREPAAQAPVKLSLNLLASSDPPEAASWLLCEVSGFSPPNILLMWLEDQREVNTSGFAPARPPPQPGSTTFWAWSVLRVPAPPSPQPATYTCVVSHEDSRTLLNASRSLEVSYVTDH

SEQ ID NO: 75 - protein, 357 aa, Artificial Sequence
  tEGFR
MLLLVTSLLLCELPHPAFLLIPRKVCNGIGIGEFKDSLSINATNIKHFKNCTSISGDLHILPVAFRGDSFTHTPPLDPQELDILKTVKEITGFLLIQAWPENRTDLHAFENLEIIRGRTKQHGQFSLAVVSLNITSLGLRSLKEISDGDVIISGNKNLCYANTINWKKLFGTSGQKTKIISNRGENSCKATGQVCHALCSPEGCWGPEPRDCVSCRNVSRGRECVDKCNLLEGEPREFVENSECIQCHPECLPQAMNITCTGRGPDNCIQCAHYIDGPHCVKTCPAGVMGENNTLVWKYADAGHVCHLCHPNCTYGCTGPGLEGCPTNGPKIPSIATGMVGALLLLLVVALGIGLFM

SEQ ID NO: 76 - protein, 24 aa, Artificial Sequence
  T2A
LEGGGEGRGSLLTCGDVEENPGPR

SEQ ID NO: 77 - protein, 27 aa, Homo sapiens
  misc_feature: CD28 (amino acids 153-179 of Accession No. P10747)
FWVLVVVGGVLACYSLLVTVAFIIFWV

SEQ ID NO: 78 - protein, 66 aa, Homo sapiens
  misc_feature: CD28 (amino acids 114-179 of Accession No. P10747)
IEVMYPPPYLDNEKSNGTIIHVKGKHLCPSPLFPGPSKPFWVLVVVGGVLACYSLLVTVAFIIFWV

SEQ ID NO: 79 - protein, 41 aa, Homo sapiens
  misc_feature: CD28 (amino acids 180-220 of P10747)
RSKRSRLLHSDYMNMTPRRPGPTRKHYQPYAPPRDFAAYRS

SEQ ID NO: 80 - protein, 41 aa, Artificial Sequence
  CD28 (LL to GG)
RSKRSRGGHSDYMNMTPRRPGPTRKHYQPYAPPRDFAAYRS

SEQ ID NO: 81 - protein, 42 aa, Homo sapiens
  misc_feature: 4-1BB (amino acids 214-255 of Q07011.1)
KRGRKKLLYIFKQPFMRPVQTTQEEDGCSCRFPEEEEGGCEL

SEQ ID NO: 82 - protein, 112 aa, Artificial Sequence
  CD3 zeta
RVKFSRSADAPAYQQGQNQLYNELNLGRREEYDVLDKRRGRDPEMGGKPRRKNPQEGLYNELQKDKMAEAYSEIGMKGERRRGKGHDGLYQGLSTATKDTYDALHMQALPPR

SEQ ID NO: 83 - protein, 112 aa, Artificial Sequence
  CD3 zeta
RVKFSRSAEPPAYQQGQNQLYNELNLGRREEYDVLDKRRGRDPEMGGKPRRKNPQEGLYNELQKDKMAEAYSEIGMKGERRRGKGHDGLYQGLSTATKDTYDALHMQALPPR

SEQ ID NO: 84 - protein, 112 aa, Artificial Sequence
  CD3 zeta
RVKFSRSADAPAYKQGQNQLYNELNLGRREEYDVLDKRRGRDPEMGGKPRRKNPQEGLYNELQKDKMAEAYSEIGMKGERRRGKGHDGLYQGLSTATKDTYDALHMQALPPR

SEQ ID NO: 85 - DNA, 33 bp, Homo sapiens
  misc_feature: Epo HRE
gccctacgtgctgtctcacacagcctgtctgac

SEQ ID NO: 86 - DNA, 35 bp, Homo sapiens
  misc_feature: VEGF-A HRE
ccacagtgcatacgtgggctccaacaggtcctctt

SEQ ID NO: 87 - DNA, 24 bp, Homo sapiens
  misc_feature: PGK1 HRE
gacgtgacaaacgaagccgacgtc

SEQ ID NO: 88 - DNA, 24 bp, Homo sapiens
  misc_feature: LdhA HRE
acacgtgggttcccgcacgtccgc

SEQ ID NO: 89 - DNA, 19 bp, Homo sapiens
  misc_feature: ALDA HRE
gacgtgactcggaccacat

SEQ ID NO: 90 - DNA, 31 bp, Homo sapiens
gcccacacgctcggtgcgtgcccagttgaac

SEQ ID NO: 91 - DNA, 10 bp, Artificial Sequence
  Exemplary CArG
ccttatttgg

SEQ ID NO: 92 - DNA, 50 bp, Artificial Sequence
  Synthetic CArG sequence-containing promoter
cgcgtgatatccttatttggccttatttggccttatttggccttatttgg

SEQ ID NO: 93 - DNA, 70 bp, Artificial Sequence
  Synthetic CArG sequence-containing promoter
cgcgtgatatccttatttggccttatttggccttatttggccttatttggccttatttggccttatttgg

SEQ ID NO: 94 - DNA, 90 bp, Artificial Sequence
  Synthetic CArG sequence-containing promoter
cgcgtgatatccttatttggccttatttggccttatttggccttatttggccttatttggccttatttggccttatttggccttatttgg

SEQ ID NO: 95 - DNA, 110 bp, Artificial Sequence
  Synthetic CArG sequence-containing promoter
cgcgtgatatccttatttggccttatttggccttatttggccttatttggccttatttggccttatttggccttatttggccttatttggccttatttggccttatttgg

SEQ ID NO: 96 - protein, 18 aa, Artificial Sequence
  T2A
EGRGSLLTCGDVEENPGP

SEQ ID NO: 97 - protein, 22 aa, Artificial Sequence
  P2A
GSGATNFSLLKQAGDVEENPGP

SEQ ID NO: 98 - protein, 19 aa, Artificial Sequence
  P2A
ATNFSLLKQAGDVEENPGP

SEQ ID NO: 99 - protein, 20 aa, Artificial Sequence
  E2A
QCTNYALLKLAGDVESNPGP

SEQ ID NO: 100 - protein, 22 aa, Artificial Sequence
  F2A
VKQTLNFDLLKLAGDVESNPGP

SEQ ID NO: 101 - protein, 335 aa, Artificial Sequence
  tEGFR
RKVCNGIGIGEFKDSLSINATNIKHFKNCTSISGDLHILPVAFRGDSFTHTPPLDPQELDILKTVKEITGFLLIQAWPENRTDLHAFENLEIIRGRTKQHGQFSLAVVSLNITSLGLRSLKEISDGDVIISGNKNLCYANTINWKKLFGTSGQKTKIISNRGENSCKATGQVCHALCSPEGCWGPEPRDCVSCRNVSRGRECVDKCNLLEGEPREFVENSECIQCHPECLPQAMNITCTGRGPDNCIQCAHYIDGPHCVKTCPAGVMGENNTLVWKYADAGHVCHLCHPNCTYGCTGPGLEGCPTNGPKIPSIATGMVGALLLLLVVALGIGLFM

SEQ ID NO: 102 - DNA, 1668 bp, Artificial Sequence
  Sc IL-12 G4S(3)
gctagcgccaccatgcccctgctgctgctgctgcctctgctgtgggctggcgcactggccatctgggagctgaagaaagacgtgtacgtggtcgaactggactggtatcctgatgccccaggagagatggtggtcctgacttgcgacacccccgaggaagatggcatcacttggaccctggatcagagctccgaggtgctgggaagcggcaaaacactgactattcaggtcaaggaattcggggacgctggacagtacacatgtcacaagggaggagaggtgctgagccactccctgctgctgctgcataagaaagaagacggcatctggagcactgacattctgaaagatcagaaggagccaaagaacaaaaccttcctgcgctgcgaagcaaaaaattatagcggccggttcacctgttggtggctgaccacaatcagcacagatctgactttttccgtgaagtctagtagggggtcaagcgacccacagggagtcacatgcggagcagctactctgtccgccgagcgggtgagaggagataacaaggagtacgaatattcagtcgagtgccaggaagacagcgcatgtcctgcagccgaggaatctctgccaatcgaagtgatggtcgatgccgtgcacaagctgaaatacgaaaactacacatcctctttctttatccgagacatcatcaagccagatccccctaagaacctgcagctgaaacccctgaagaattctcgccaggtggaggtcagttgggaatacccagacacctggagcacaccccattcatatttcagcctgactttttgcgtgcaggtccagggcaagagtaaaagagagaagaaagacagggtgttcactgataaaaccagcgccacagtcatctgtcggaagaacgcctctattagtgtgcgagctcaggatcggtactatagttcaagctggtccgaatgggcttctgtgccttgtagtggaggaggaggaagcggaggaggaggatccggaggaggcgggtctagaaatctgcctgtggcaaccccagaccccggcatgttcccatgcctgcaccattcccagaacctgctgcgggcagtgtctaatatgctgcagaaggccagacagaccctggagttttacccctgtacatccgaggaaatcgaccacgaggatattaccaaggataaaacctctacagtggaagcttgcctgcctctggagctgacaaagaacgaatcatgtctgaatagcagggagacttccttcatcaccaacggctcttgcctggccagtcgcaagaccagcttcatgatggctctgtgcctgtcctctatctacgaggacctgaagatgtatcaggtggaattcaaaaccatgaacgccaagctgctgatggaccctaaaaggcagatctttctggatcagaatatgctggctgtgattgacgagctgatgcaggcactgaacttcaatagcgaaacagtcccccagaagagttcactggaggaacctgatttctacaagactaaaatcaagctgtgcattctgctgcacgcttttaggatccgcgcagtgaccattgaccgcgtcatgagttatctgaatgcctcacaccatcaccatcaccattggtcccatccacagtttgagaagtgataactcgag

SEQ ID NO: 103 - DNA, 1683 bp, Artificial Sequence
  Sc IL-12 HBP BMP4
gctagcgccaccatgcccctgctgctgctgctgcctctgctgtgggctggcgcactggccatctgggagctgaagaaagacgtgtacgtggtcgaactggactggtatcctgatgccccaggggagatggtggtcctgacttgcgacacccccgaggaagatggaatcacttggaccctggatcagagctccgaggtgctggggtccggaaaaacactgactattcaggtcaaggaattcggcgacgctgggcagtacacatgtcacaagggaggagaggtgctgagccactccctgctgctgctgcataagaaagaagacggaatctggtctactgacattctgaaagatcagaaggagcctaagaacaaaaccttcctgcggtgcgaagcaaaaaattatagcggccggttcacctgttggtggctgaccacaatctctacagatctgacttttagtgtgaagtctagtaggggctcaagcgacccacagggagtcacatgcggagcagctactctgagcgccgagagggtgcgcggggataacaaggagtacgaatattccgtcgagtgccaggaagactctgcatgtcctgcagccgaggaatccctgccaatcgaagtgatggtcgatgccgtgcacaagctgaaatacgaaaactacacatcctctttctttattagggacatcatcaagccagatccccctaagaacctgcagctgaaacccctgaagaattcacgccaggtggaggtcagctgggaatacccagacacctggagcacaccccattcatatttcagcctgactttttgcgtgcaggtccagggcaagagcaaacgcgagaagaaagaccgagtgttcactgataaaacctccgctacagtcatctgccgcaagaacgcctctattagtgtgagagctcaggataggtactatagttcaagctggtccgaatgggcatctgtgccatgcagtggaggaggaggaagccggaagaaaaaccctaattgtcggagacacggcgggggaggctccagaaatctgcctgtggctaccccagaccccgggatgttcccatgcctgcaccatagtcagaacctgctgagggcagtgtcaaatatgctgcagaaggcccgccagaccctggagttttacccatgtacatctgaggaaatcgaccacgaggatattaccaaggataaaaccagtacagtggaagcctgcctgcccctggagctgacaaagaacgaatcatgtctgaatagccgagagacttccttcatcaccaacggctcttgcctggccagtcgcaagaccagcttcatgatggctctgtgcctgtcctctatctacgaggacctgaagatgtatcaggtggaattcaaaaccatgaacgccaagctgctgatggaccccaaacggcagatctttctggatcagaatatgctggctgtgattgacgagctgatgcaggcactgaacttcaattctgaaacagtcccccagaagagttcactggaggaacctgatttctacaagactaaaatcaagctgtgcattctgctgcacgcttttcgaatccgggcagtgaccattgacagagtcatgagctatctgaatgcctcccaccatcaccatcaccattggagccatcctcagtttgagaagtgataactcgag

SEQ ID NO: 104 - DNA, 1698 bp, Artificial Sequence
  Sc IL-12 HBP FBN
gctagcgccaccatgcccctgctgctgctgctgcctctgctgtgggctggcgcactggccatctgggagctgaagaaagacgtgtacgtggtcgaactggactggtatcctgatgccccaggggagatggtggtcctgacttgcgacacccccgaggaagatggaatcacttggaccctggatcagagctccgaggtgctggggagcggaaaaacactgactattcaggtcaaggaattcggcgacgctgggcagtacacatgtcacaagggaggagaggtgctgagccactccctgctgctgctgcataagaaagaagacgggatctggtctacagacattctgaaagatcagaaggagcctaagaacaaaactttcctgcgctgcgaagcaaaaaattatagcggccggttcacctgttggtggctgaccacaatctctacagatctgacttttagtgtgaagtctagtaggggatcaagcgacccacagggagtcacatgcggagcagctactctgagcgccgagcgggtgagaggcgataacaaggagtacgaatatagtgtcgagtgccaggaagactcagcatgtcctgcagccgaggaatccctgccaatcgaagtgatggtcgatgccgtgcacaagctgaaatacgaaaactacacatcctctttctttattcgggacatcatcaagccagatccccctaagaacctgcagctgaaacccctgaagaattcaagacaggtggaggtcagctgggaatacccagacacctggtccacaccccattcatatttcagcctgaccttttgcgtgcaggtccagggcaagtctaaaagagagaagaaagacagggtgttcactgataaaaccagtgctacagtcatctgtagaaagaacgcctctattagtgtgcgagctcaggatcggtactatagttcaagctggtccgagtgggcatctgtgccctgtagtggaggcgggggatccaaaaacaatcagaagtctgaacctctgatcggccggaagaaaactggcgggggaggcagcagaaatctgcctgtggctaccccagatcccgggatgttcccatgcctgcaccatagccagaacctgctgagggcagtgtccaatatgctgcagaaggcccgccagaccctggagttttacccatgtacaagcgaggaaatcgaccacgaggatattactaaggacaaaacctccacagtggaagcctgcctgcccctggagctgaccaagaacgaatcatgtctgaatagccgagagacttccttcatcaccaacggctcttgcctggccagtcgcaagaccagcttcatgatggctctgtgcctgtcctctatctacgaggacctgaagatgtatcaggtggaattcaaaactatgaacgccaagctgctgatggaccccaaaaggcagatctttctggatcagaatatgctggctgtgattgacgagctgatgcaggcactgaacttcaattctgaaaccgtcccccagaagagttcactggaggaacctgatttctacaagacaaaaatcaagctgtgcattctgctgcacgcttttaggatccgcgcagtgaccattgaccgcgtcatgagctatctgaatgcctcccaccatcaccatcaccattggagccatcctcagtttgagaagtgataactcgag

SEQ ID NO: 105 - DNA, 1701 bp, Artificial Sequence
  Sc IL-12 HGFBP
gctagcgccaccatgcccctgctgctgctgctgcctctgctgtgggctggcgcactggccatctgggagctgaagaaagacgtgtacgtggtcgaactggactggtatcctgatgccccaggggagatggtggtcctgacttgcgacacccccgaggaagatggaatcacttggaccctggatcagagctccgaggtgctggggtccggaaaaacactgactattcaggtcaaggaattcggcgacgctgggcagtacacatgtcacaagggaggagaggtgctgagccactccctgctgctgctgcataagaaagaagacgggatctggtctactgacattctgaaagatcagaaggagccaaagaacaaaaccttcctgcgctgcgaagcaaaaaattatagcggccggttcacctgttggtggctgaccacaatctctacagatctgacttttagtgtgaagtctagtaggggctcaagcgacccacagggagtcacatgcggagcagctactctgagcgccgagcgggtgagaggggataacaaggagtacgaatattccgtcgagtgccaggaagactctgcatgtcctgcagccgaggaatccctgccaatcgaagtgatggtcgatgccgtgcacaagctgaaatacgaaaactacacatcctctttctttattcgggacatcatcaagccagatccccctaagaacctgcagctgaaacccctgaagaattcaagacaggtggaggtcagctgggaatacccagacacctggagcacaccccattcatatttcagcctgactttttgcgtgcaggtccagggcaagagcaaaagagagaagaaagacagggtgttcactgataaaacctccgctacagtcatctgcagaaagaacgcctctattagtgtgcgagctcaggatcggtactatagttcaagctggtccgaatgggcatctgtgccttgtagtggaggcgggggaagcgtgtggaactgggtctgctttagggacgtgggatgtgattgggtcctgggaggaggaggctcccgcaatctgcctgtggctaccccagatcccggcatgttcccatgcctgcaccatagtcagaacctgctgcgggcagtgtcaaatatgctgcagaaggccagacagaccctggagttttacccctgtacatctgaggaaatcgaccacgaggatattaccaaggacaaaaccagtacagtggaagcctgcctgcctctggagctgacaaagaacgaatcatgtctgaatagccgagagacttccttcatcaccaacggctcttgcctggccagtcgcaagaccagcttcatgatggctctgtgcctgtcctctatctacgaggacctgaagatgtatcaggtggaattcaaaaccatgaacgccaagctgctgatggaccctaaaaggcagatctttctggatcagaatatgctggctgtgattgacgagctgatgcaggcactgaacttcaattctgaaacagtgccccagaagagttcactggaggaacctgatttctacaagactaaaatcaagctgtgcattctgctgcacgcttttaggatccgcgcagtgaccattgaccgcgtcatgagctatctgaatgcctcccaccatcaccatcaccattggagccatccacagtttgagaagtgataactcgag

SEQ ID NO: 106 - DNA, 1677 bp, Artificial Sequence
  Sc IL-12 EGFRBP
gctagcgccaccatgcccctgctgctgctgctgcctctgctgtgggctggcgcactggccatctgggagctgaagaaagacgtgtacgtggtcgaactggactggtatcctgatgccccaggggagatggtggtcctgacttgcgacacccccgaggaagatggaatcacttggaccctggatcagagctccgaggtgctggggagcggaaaaacactgactattcaggtcaaggaattcggcgacgctgggcagtacacatgtcacaagggcggggaggtgctgtctcacagtctgctgctgctgcataagaaagaagacggaatctggtctactgacattctgaaagatcagaaggagcctaagaacaaaaccttcctgcgctgcgaagcaaaaaattatagcggccggttcacctgttggtggctgaccacaatctcaacagatctgacttttagcgtgaagtctagtaggggctcaagcgacccacagggagtcacatgcggagcagctactctgagcgccgagcgggtgagaggggataacaaggagtacgaatatagtgtcgagtgccaggaagactcagcatgtcctgcagccgaggaatccctgccaatcgaagtgatggtcgatgccgtgcacaagctgaaatacgaaaactacacatcctctttctttatccgagacatcatcaagccagatccccctaagaacctgcagctgaaacccctgaagaattcccgccaggtggaggtctcttgggaatacccagacacctggtccacaccccattcctatttctctctgactttttgcgtgcaggtccagggcaagtctaaaagagagaagaaagacagggtgttcactgataaaaccagtgctacagtcatctgccggaagaacgcctcaattagcgtgcgagctcaggaccggtactatagttcaagctggagtgaatgggcatcagtgccatgcagcggaggaggaggatcctctgtggataaccctcacgtctgtggcggaggaggcagcagaaatctgcctgtggctaccccagaccccgggatgttcccatgcctgcaccatagccagaacctgctgcgggcagtgtccaatatgctgcagaaggccagacagaccctggagttttacccatgtacaagcgaggaaatcgaccacgaggatattaccaaggataaaacctccacagtggaagcctgcctgcccctggagctgacaaagaacgaatcctgtctgaattctagggagactagtttcatcaccaacggctcatgcctggccagccgcaaaacttcctttatgatggctctgtgcctgagttcaatctacgaggacctgaagatgtatcaggtggaattcaaaaccatgaacgccaagctgctgatggaccccaaaaggcagatctttctggatcagaatatgctggctgtgattgacgagctgatgcaggcactgaacttcaattctgaaacagtcccccagaagagctccctggaggaacctgatttctacaagactaaaatcaagctgtgcattctgctgcacgcttttaggatccgcgcagtgaccattgaccgcgtcatgtcttatctgaatgccagtcaccatcaccatcaccattggagccatcctcagtttgagaagtgataactcgag

SEQ ID NO: 107 - DNA, 2394 bp, Artificial Sequence
  Sc IL-12 anti-EPCAM
gctagcgccaccatgcctctgctgctgctgctgccactgctgtgggctggcgcactggccatctgggagctgaagaaagacgtgtacgtggtcgaactggactggtatcccgatgctcctggggagatggtggtcctgacatgcgacactcccgaggaagatggaatcacatggactctggatcagagctccgaggtcctgggaagcggcaaaaccctgacaattcaggtgaaggaattcggggacgccggacagtacacatgtcacaagggcggggaggtgctgtctcacagtctgctgctgctgcataagaaagaagacgggatctggtctaccgacattctgaaagatcagaaggagcccaagaacaaaacattcctgaggtgcgaagccaaaaattatagcggacgctttacctgttggtggctgaccacaatcagtaccgatctgacattttcagtcaagtctagtcggggctcaagcgaccctcagggagtgacatgcggagcagctactctgtctgccgagcgggtcagaggggataacaaggagtacgaatattctgtggagtgccaggaagacagtgcttgtccagcagccgaggaaagcctgcccatcgaggtcatggtggatgcagtgcacaagctgaaatacgaaaactacacatcctctttctttattcgggacatcatcaagccagatccccctaagaacctgcagctgaaacccctgaagaatagcagacaggtcgaggtgtcctgggaataccccgacacttggagcacccctcatagttatttctcactgaccttttgcgtccaggtgcagggcaagtctaaaagagagaagaaagacagggtcttcacagataagaccagcgccaccgtgatctgtagaaagaacgcatcaattagcgtgcgagcccaggatcggtactatagttcaagctggagcgagtgggcctccgtgccatgctctggaggaggaggatcacaggtccagctggtgcagagcggagcagaagtgaagaaacccggctcctctgtcaaagtgagttgtaaggcctcaggcgggacttttagttcatacgcaatctctgtggtcgtgaggcaggcaccaggacagggactggagtggatgggaggcatcattcctatcttcggcaccgccaactacgctcagaagtttcaggggcgcgtgactattaccgccgatgagtccacatctactgcttatatggagctgagctccctgagaagcgaagacaccgccgtgtactattgcgcaaggggcctgctgtggaattactggggccaggggacactggtcaccgtgagcagcaaactgagtggaagcgccagcgcccctaagctggaggaaggagagttcagtgaagcccgggtcgagactaccctgacccagtcccctgctacactgtccgtgtctccaggagaacgcgctacactgagctgtcgagcaagtcagtcagtgtcaagcaatctggctgtcgtgtaccagcagaagccaggccaggcacccagactgctgatctatggggcaagcacccgggccacaggaattccagctagattcagcggatccggctctgggaccgagtttaccctgacaatctcctctctgcagtccgaagacttcgccgtgtactattgccagcagtacaacaattggccacccgggttcacttttggacccggcaccaaagtcgatattaagggaggaggagggtcccggaacctgcctgtggcaactcctgacccaggcatgttcccatgcctgcaccattcccagaacctgctgcgagccgtgagcaatatgctgcagaaagcacggcagacactggagttttatccttgtactagcgaggaaatcgaccacgaggatattacaaaggataaaacttccaccgtggaagcctgcctgccactggagctgactaagaacgaaagctgtctgaattcccgcgagacttctttcatcaccaatggcagttgcctggcatcacgaaaaaccagctttatgatggccctgtgcctgagttcaatctacgaggacctgaagatgtatcaggtggaattcaaaacaatgaacgccaagctgctgatggaccctaaaaggcagatctttctggatcagaatatgctggccgtgattgacgagctgatgcaggctctgaacttcaatagcgaaactgtgccccagaagagctccctggaggaacctgatttctacaagaccaaaatcaagctgtgcattctgctgcacgcctttaggatccgcgctgtcaccattgaccgcgtgatgtcctatctgaacgcctctcaccatcaccatcaccattggtcccatccacagtttgagaagtgataactcgag

SEQ ID NO: 108 - protein, 12 aa, Artificial Sequence
  EGFR binding peptide
YHWYGYTPQNVI

SEQ ID NO: 109 - protein, 12 aa, Artificial Sequence
  EGFR binding peptide
YRWYGYTPQNVI

SEQ ID NO: 110 - protein, 6 aa, Artificial Sequence
  VEGFR3 binding peptide
PCAIWF

SEQ ID NO: 111 - protein, 6 aa, Artificial Sequence
  VEGFR3 binding peptide
WVCSGG

SEQ ID NO: 112 - protein, 9 aa, Artificial Sequence
  NGR motif
NGRNGRNGR

SEQ ID NO: 113 - protein, 9 aa, Artificial Sequence
  RGD motif
RGDRGDRGD

SEQ ID NO: 114 - protein, 10 aa, Artificial Sequence
  NG2 proteoglycan binding peptide
TAASGVRSMH

SEQ ID NO: 115 - protein, 10 aa, Artificial Sequence
  NG2 proteoglycan binding peptide
LTLRWVGLMS

SEQ ID NO: 116 - protein, 25 aa, Artificial Sequence
  HER2 binding peptide
NKFNKGMRYWGALGGNGKRGIRGYM

SEQ ID NO: 117 - protein, 9 aa, Artificial Sequence
  EPCAM binding peptide
YEVHTYYLD

SEQ ID NO: 118 - protein, 21 aa, Artificial Sequence
  VEGFR binding peptide
ITMQIMRIKPHQGQHIGEMSF